European Patent Application EP 4 516 931 A1, published March 5, 2025. Title: 핫스팟 유래 펩타이드-핵산 하이브리드 분자를 포함하는, 변이 코로나 바이러스에 의한 감염증 치료용 조성물. Applicant: POSTECH Research and Business Development Foundation. The sequence listing filed with the application follows.

SEQUENCE LISTING (23 sequences)

SEQ ID NO: 1 - DNA, 15 bp, synthetic construct
  source 1..15: mol_type = other DNA
ggaagagatggcgac

SEQ ID NO: 2 - DNA, 15 bp, synthetic construct
  source 1..15: mol_type = other DNA
ccatcaggatcagct

SEQ ID NO: 3 - DNA, 70 bp, synthetic construct
  source 1..70: mol_type = other DNA
ggaagagatggcgacnnnnnnnnnnnnnnnnnnnnnnnnnnnnnnnnnnnnnnnnagctgatcctgatgg

SEQ ID NO: 4 - DNA, 92 bp, synthetic construct
  source 1..92: mol_type = other DNA
aatgatacggcgaccaccgagatctacacttggtgagacactctttccctacacgacgctcttccgatctnnnnnnnggaagagatggcgac

SEQ ID NO: 5 - DNA, 87 bp, synthetic construct
  source 1..87: mol_type = other DNA
caagcagaagacggcatacgagatgttcaggtctgactggagttcagacgtgtgctcttccgatctnnnnnnccatcaggatcagct

SEQ ID NO: 6 - DNA, 65 bp, synthetic construct
  source 1..65: mol_type = other DNA
ggaagagatggcgacctccacaaccgctgatcgacgcagatcttgtgggtagctgatcctgatgg

SEQ ID NO: 7 - DNA, 60 bp, synthetic construct
  source 1..60: mol_type = other DNA
ggaagagatggcgacacgcaatcgtgggttggggatataatggtaagctgatcctgatgg

SEQ ID NO: 8 - DNA, 60 bp, synthetic construct; identical to SEQ ID NO: 7
  source 1..60: mol_type = other DNA

SEQ ID NO: 9 - DNA, 60 bp, synthetic construct
  source 1..60: mol_type = other DNA
ggaagagatggcgaccacaccaaatctgagtctaccccatgaaggagctgatcctgatgg

SEQ ID NO: 10 - DNA, 51 bp, synthetic construct
  source 1..51: mol_type = other DNA
cagcaccgaccttgtgctttgggagtgctggtccaagggcgttaatggaca

SEQ ID NO: 11 - DNA, 46 bp, synthetic construct
  source 1..46: mol_type = other DNA
cgcagcacccaagaacaaggactgcttaggattgcgataggttcgg

SEQ ID NO: 12 - DNA, 40 bp, synthetic construct
  source 1..40: mol_type = other DNA
tcgagtggcttgtttgtaatgtagggttccggtcgtgggt

SEQ ID NO: 13 - DNA, 60 bp, synthetic construct; identical to SEQ ID NO: 7
  source 1..60: mol_type = other DNA
  misc_difference 2..5: note = 2'-O-Methyl modified
  misc_difference 56..58: note = 2'-O-Methyl modified
  misc_difference 59: note = 2'-F modified

SEQ ID NO: 14 - DNA, 60 bp, synthetic construct; identical to SEQ ID NO: 7
  source 1..60: mol_type = other DNA
  misc_difference 1..4: note = Phosphorothioate modified
  misc_difference 56..59: note = Phosphorothioate modified

SEQ ID NO: 15 - protein, 7 aa, synthetic construct
LGKGDFR

SEQ ID NO: 16 - DNA, 35 bp, synthetic construct
  source 1..35: mol_type = other DNA
ctccacaaccgctgatcgacgcagatcttgtgggt

SEQ ID NO: 17 - DNA, 34 bp, synthetic construct
  source 1..34: mol_type = other DNA
ctccacaaccgctgatcgacgcagatcttgtggt

SEQ ID NO: 18 - DNA, 30 bp, synthetic construct
  source 1..30: mol_type = other DNA
acgcaatcgtgggttggggatataatggta

SEQ ID NO: 19 - DNA, 30 bp, synthetic construct
  source 1..30: mol_type = other DNA
acgcaatcgtgggttggggacataatggta

SEQ ID NO: 20 - DNA, 29 bp, synthetic construct
  source 1..29: mol_type = other DNA
acgcaatcgtgggttgggatataatggta

SEQ ID NO: 21 - DNA, 30 bp, synthetic construct
  source 1..30: mol_type = other DNA
cacaccaaatctgagtctaccccatgaagg

SEQ ID NO: 22 - DNA, 30 bp, synthetic construct
  source 1..30: mol_type = other DNA
cacaccaaatctgagtctaccctatgaagg

SEQ ID NO: 23 - protein, 219 aa, synthetic construct
RVQPTESIVRFPNITNLCPFGEVFNATRFASVYAWNRKRISNCVADYSVLYNSASFSTFKCYGVSPTKLNDLCFTNVYADSFVIRGDEVRQIAPGQTGKIADYNYKLPDDFTGCVIAWNSNNLDSKVGGNYNYLYRLFRKSNLKPFERDISTEIYQAGSTPCNGVEGFNCYFPLQSYGFQPTNGVGYQPYRVVVLSFELLHAPATVCGPKKSTNLVKNK